European Patent Specification EP 3 481 867 B1, published September 4, 2024. Title: PROGRAMMED DEATH 1 LIGAND 1 (PD-L1) BINDING PROTEINS AND METHODS OF USE THEREOF. Applicant: IOVANCE BIOTHERAPEUTICS Rabinovich, Brian Martin-Orozco, Natalia Radvanyi, Laszlo. The sequence listing filed with the application follows.

SEQUENCE LISTING (42 sequences)

SEQ ID NO: 1 - protein, 108 aa, Artificial Sequence
  synthetic sequence
SYVLTQPPSVSVAPGQTARITCGGNNIGRKIVHWYQQRPGQAPVLVIYYDTDRPAGIPERFSGSNSGNMATLTISTVGAGDEADYYCQVWDTGSDHVVFGGGTKLTVL

SEQ ID NO: 2 - protein, 6 aa, Artificial Sequence
  synthetic sequence
NIGRKI

SEQ ID NO: 3 - protein, 3 aa, Artificial Sequence
  synthetic sequence
YDT

SEQ ID NO: 4 - protein, 11 aa, Artificial Sequence
  synthetic sequence
QVWDTGSDHVV

SEQ ID NO: 5 - protein, 122 aa, Artificial Sequence
  synthetic sequence
EVQLVESGGGLVQPGGSLRLSCAASGFTFSNYAMSWVRQAPGKGLEWVSTISGSGGTTYYADSVKGRFTISRDNSKNTLYLQMNSLRVEDTAVYYCAKDWFRSSSPDAFDIWGQGTTVTVSA

SEQ ID NO: 6 - protein, 8 aa, Artificial Sequence
  synthetic sequence
GFTFSNYA

SEQ ID NO: 7 - protein, 8 aa, Artificial Sequence
  synthetic sequence
ISGSGGTT

SEQ ID NO: 8 - protein, 15 aa, Artificial Sequence
  synthetic sequence
AKDWFRSSSPDAFDI

SEQ ID NO: 9 - protein, 110 aa, Artificial Sequence
  synthetic sequence
NFMLTQPHSVSESLGKTVTISCTGSSGSIARKFVQWYQQRPGSSPTTVIYENNQRPSGVSDRFSGSIGSSSNSASLTISGLKTEDEADYYCQSYDSSNVVFGGGTKVTVL

SEQ ID NO: 10 - protein, 8 aa, Artificial Sequence
  synthetic sequence
SGSIARKF

SEQ ID NO: 11 - protein, 3 aa, Artificial Sequence
  synthetic sequence
ENN

SEQ ID NO: 12 - protein, 9 aa, Artificial Sequence
  synthetic sequence
QSYDSSNVV

SEQ ID NO: 13 - protein, 123 aa, Artificial Sequence
  synthetic sequence
QVQLQESGGGLVKPGGSLRLSCAASGFTFSSYSMNWVRQAPGKGLEWVSGINTAGDTHYPESVKGRFTISRDNARNSLNLQMNSLRAEDTAVYYCVRERVEREYSGYDAFDIWGQGTTVTVSA

SEQ ID NO: 14 - protein, 8 aa, Artificial Sequence
  synthetic sequence
GFTFSSYS

SEQ ID NO: 15 - protein, 7 aa, Artificial Sequence
  synthetic sequence
INTAGDT

SEQ ID NO: 16 - protein, 17 aa, Artificial Sequence
  synthetic sequence
VRERVEREYSGYDAFDI

SEQ ID NO: 17 - protein, 248 aa, Artificial Sequence
  synthetic sequence
EVQLVESGGGLVQPGGSLRLSCAASGFTFSNYAMSWVRQAPGKGLEWVSTISGSGGTTYYADSVKGRFTISRDNSKNTLYLQMNSLRVEDTAVYYCAKDWFRSSSPDAFDIWGQGTTVTVSAGGGGSGGGGSGGGGSGAPSYVLTQPPSVSVAPGQTARITCGGNNIGRKIVHWYQQRPGQAPVLVIYYDTDRPAGIPERFSGSNSGNMATLTISTVGAGDEADYYCQVWDTGSDHVVFGGGTKLTVL

SEQ ID NO: 18 - protein, 511 aa, Artificial Sequence
  synthetic sequence
MGSTAILALLLAVLQGVSAEVQLVESGGGLVQPGGSLRLSCAASGFTFSNYAMSWVRQAPGKGLEWVSTISGSGGTTYYADSVKGRFTISRDNSKNTLYLQMNSLRVEDTAVYYCAKDWFRSSSPDAFDIWGQGTTVTVSAGGGGSGGGGSGGGGSGAPSYVLTQPPSVSVAPGQTARITCGGNNIGRKIVHWYQQRPGQAPVLVIYYDTDRPAGIPERFSGSNSGNMATLTISTVGAGDEADYYCQVWDTGSDHVVFGGGTKLTVLGPRANFVYKSGPRPKSCDKTHTCPPCPAPELLGGPSVFLFPPKPKDTLMISRTPEVTCVVVDVSHEDPEVKFNWYVDGVEVHNAKTKPREEQYNSTYRVVSVLTVLHQDWLNGKEYKCKVSNKALPAPIEKTISKAKGQPREPQVYTLPPSREEMTKNQVSLTCLVKGFYPSDIAVEWESNGQPENNYKTTPPVLDSDGSFFLYSKLTVDKSRWQQGNVFSCSVMHEALHNHYTQKSLSLSPGK

SEQ ID NO: 19 - protein, 251 aa, Artificial Sequence
  synthetic sequence
QVQLQESGGGLVKPGGSLRLSCAASGFTFSSYSMNWVRQAPGKGLEWVSGINTAGDTHYPESVKGRFTISRDNARNSLNLQMNSLRAEDTAVYYCVRERVEREYSGYDAFDIWGQGTTVTVSAGGGGSGGGGSGGGGSGAPNFMLTQPHSVSESLGKTVTISCTGSSGSIARKFVQWYQQRPGSSPTTVIYENNQRPSGVSDRFSGSIGSSSNSASLTISGLKTEDEADYYCQSYDSSNVVFGGGTKVTVL

SEQ ID NO: 20 - protein, 514 aa, Artificial Sequence
  synthetic sequence
MGSTAILALLLAVLQGVSAQVQLQESGGGLVKPGGSLRLSCAASGFTFSSYSMNWVRQAPGKGLEWVSGINTAGDTHYPESVKGRFTISRDNARNSLNLQMNSLRAEDTAVYYCVRERVEREYSGYDAFDIWGQGTTVTVSAGGGGSGGGGSGGGGSGAPNFMLTQPHSVSESLGKTVTISCTGSSGSIARKFVQWYQQRPGSSPTTVIYENNQRPSGVSDRFSGSIGSSSNSASLTISGLKTEDEADYYCQSYDSSNVVFGGGTKVTVLGPRANFVYKSGPRPKSCDKTHTCPPCPAPELLGGPSVFLFPPKPKDTLMISRTPEVTCVVVDVSHEDPEVKFNWYVDGVEVHNAKTKPREEQYNSTYRVVSVLTVLHQDWLNGKEYKCKVSNKALPAPIEKTISKAKGQPREPQVYTLPPSREEMTKNQVSLTCLVKGFYPSDIAVEWESNGQPENNYKTTPPVLDSDGSFFLYSKLTVDKSRWQQGNVFSCSVMHEALHNHYTQKSLSLSPGK

SEQ ID NO: 21 - protein, 290 aa, Artificial Sequence
  synthetic sequence
MRIFAVFIFMTYWHLLNAFTVTVPKDLYVVEYGSNMTIECKFPVEKQLDLAALIVYWEMEDKNIIQFVHGEEDLKVQHSSYRQRARLLKDQLSLGNAALQITDVKLQDAGVYRCMISYGGADYKRITVKVNAPYNKINQRILVVDPVTSEHELTCQAEGYPKAEVIWTSSDHQVLSGKTTTTNSKREEKLFNVTSTLRINTTTNEIFYCTFRRLDPEENHTAELVIPELPLAHPPNERTHLVILGAILLCLGVALTFIFRLRKGRMMDVKKCGIQDTNSKKQSDTHLEET

SEQ ID NO: 22 - protein, 228 aa, Artificial Sequence
  synthetic sequence
CPPCPAPEFEGGPSVFLFPPKPKDTLMETISRTPEVTCVVVDVSQEDPEVQFNWYVDGVEVHNAKTKPREEQFQSTYRVVSVLTVLHQDWLNGKEYKCKVSNKGLPSSIEKTISKAKGQPREPQVYTLPPSQEEMETTKNQVSLTCLVKGFYPSDIAVEWESNGQPENNYKTTPPVLDSDGSFFLYSRLTVDKSRWQEGNVFSCSVMETHEALHNHYTQKSLSLSLGK

SEQ ID NO: 23 - protein, 228 aa, Artificial Sequence; identical to SEQ ID NO: 22
  synthetic sequence

SEQ ID NO: 24 - protein, 46 aa, Artificial Sequence
  synthetic sequence
RSGSSRMETKQIEDKIEEILSKIYHIENEIARIKKLIGERGTSSRG

SEQ ID NO: 25 - protein, 189 aa, Artificial Sequence
  synthetic sequence
ASSIVYKKEGEQVEFSFPLAFTVEKLTGSGELWWQAERASSSKSWITFDLKNKEVSVKRVTQDPKLQMETGKKLPLHLTLPQALPQYAGSGNLTLALEAKTGKLHQEVNLVVMETRATQLQKNLTCEVWGPTSPKLMETLSLKLENKEAKVSKREKAVWVLNPEAGMETWQCLLSDSGQVLLESNIKVL

SEQ ID NO: 26 - protein, 28 aa, Artificial Sequence
  synthetic sequence
SSSSKAPPPSLPSPSRLPGPSDTPILPQ

SEQ ID NO: 27 - protein, 450 aa, Artificial Sequence
  synthetic sequence
QVQLQQSGAELARPGASVKMSCKASGYTFTRYTMHWVKQRPGQGLEWIGYINPSRGYTNYNQKFKDKATLTTDKSSSTAYMQLSSLTSEDSAVYYCARYYDDHYCLDYWGQGTTLTVSSAKTTAPSVYPLAPVCGGTTGSSVTLGCLVKGYFPEPVTLTWNSGSLSSGVHTFPAVLQSDLYTLSSSVTVTSSTWPSQSITCNVAHPASSTKVDKKIEPRPKSCDKTHTCPPCPAPELLGGPSVFLFPPKPKDTLMISRTPEVTCVVVDVSHEDPEVKFNWYVDGVEVHNAKTKPREEQYNSTYRVVSVLTVLHQDWLNGKEYKCKVSNKALPAPIEKTISKAKGQPREPQVYTLPPSRDELTKNQVSLTCLVKGFYPSDIAVEWESNGQPENNYKTTPPVLDSDGSFFLYSKLTVDKSRWQQGNVFSCSVMHEALHNHYTQKSLSLSPGK

SEQ ID NO: 28 - protein, 213 aa, Artificial Sequence
  synthetic sequence
QIVLTQSPAIMSASPGEKVTMTCSASSSVSYMNWYQQKSGTSPKRWIYDTSKLASGVPAHFRGSGSGTSYSLTISGMEAEDAATYYCQQWSSNPFTFGSGTKLEINRADTAPTVSIFPPSSEQLTSGGASVVCFLNNFYPKDINVKWKIDGSERQNGVLNSWTDQDSKDSTYSMSSTLTLTKDEYERHNSYTCEATHKTSTSPIVKSFNRNEC

SEQ ID NO: 29 - protein, 134 aa, Artificial Sequence
  synthetic sequence
MAPTSSSTKKTQLQLEHLLLDLQMILNGINNYKNPKLTRMLTFKFYMPKKATELKHLQCLEEELKPLEEVLNLAQSKNFHLRPRDLISNINVIVLELKGSETTFMCEYADETATIVEFLNRWITFCQSIISTLT

SEQ ID NO: 30 - protein, 132 aa, Artificial Sequence
  synthetic sequence
PTSSSTKKTQLQLEHLLLDLQMILNGINNYKNPKLTRMLTFKFYMPKKATELKHLQCLEEELKPLEEVLNLAQSKNFHLRPRDLISNINVIVLELKGSETTFMCEYADETATIVEFLNRWITFSQSIISTLT

SEQ ID NO: 31 - protein, 130 aa, Artificial Sequence
  synthetic sequence
MHKCDITLQEIIKTLNSLTEQKTLCTELTVTDIFAASKNTTEKETFCRAATVLRQFYSHHEKDTRCLGATAQQFHRHKQLIRFLKRLDRNLWGLAGLNSCPVKEANQSTLENFLERLKTIMREKYSKCSS

SEQ ID NO: 32 - protein, 153 aa, Artificial Sequence
  synthetic sequence
MDCDIEGKDGKQYESVLMVSIDQLLDSMKEIGSNCLNNEFNFFKRHICDANKEGMFLFRAARKLRQFLKMNSTGDFDLHLLKVSEGTTILLNCTGQVKGRKPAALGEAQPTKSLEENKSLKEQKKLNDLCFLKRLLQEIKTCWNKILMGTKEH

SEQ ID NO: 33 - protein, 115 aa, Artificial Sequence
  synthetic sequence
MNWVNVISDLKKIEDLIQSMHIDATLYTESDVHPSCKVTAMKCFLLELQVISLESGDASIHDTVENLIILANNSLSSNGNVTESGCKECEELEEKNIKEFLQSFVHIVQMFINTS

SEQ ID NO: 34 - protein, 132 aa, Artificial Sequence
  synthetic sequence
MQDRHMIRMRQLIDIVDQLKNYVNDLVPEFLPAPEDVETNCEWSAFSCFQKAQLKSANTGNNERIINVSIKKLKRKPPSTNAGRRQKHRLTCPSCDSYEKKPPKEFLERFKSLLQKMIHQHLSSRTHGSEDS

SEQ ID NO: 35 - DNA, 8449 bp, Artificial Sequence
  pLV430G (Lentiviral Vector)
cgataaccctaattcgatagcatatgcttcccgttgggtaacatatgctattgaattagggttagtctggatagtatatactactacccgggaagcatatgctacccgtttagggttcaccggtgatgccggccacgatgcgtccggcgtagaggatctaatgtgagttagctcactcattaggcaccccaggctttacactttatgcttccggctcgtatgttgtgtggaattgtgagcggataacaatttcacacaggaaacagctatgaccatgattacgccaagcgcgcaattaaccctcactaaagggaacaaaagctggagctgcaagcttaatgtagtcttatgcaatactcttgtagtcttgcaacatggtaacgatgagttagcaacatgccttacaaggagagaaaaagcaccgtgcatgccgattggtggaagtaaggtggtacgatcgtgccttattaggaaggcaacagacgggtctgacatggattggacgaaccactgaattgccgcattgcagagatattgtatttaagtgcctagctcgatacataaacgggtctctctggttagaccagatctgagcctgggagctctctggctaactagggaacccactgcttaagcctcaataaagcttgccttgagtgcttcaagtagtgtgtgcccgtctgttgtgtgactctggtaactagagatccctcagacccttttagtcagtgtggaaaatctctagcagtggcgcccgaacagggacttgaaagcgaaagggaaaccagaggagctctctcgacgcaggactcggcttgctgaagcgcgcacggcaagaggcgaggggcggcgactggtgagtacgccaaaaattttgactagcggaggctagaaggagagagatgggtgcgagagcgtcagtattaagcgggggagaattagatcgcgatgggaaaaaattcggttaaggccagggggaaagaaaaaatataaattaaaacatatagtatgggcaagcagggagctagaacgattcgcagttaatcctggcctgttagaaacatcagaaggctgtagacaaatactgggacagctacaaccatcccttcagacaggatcagaagaacttagatcattatataatacagtagcaaccctctattgtgtgcatcaaaggatagagataaaagacaccaaggaagctttagacaagatagaggaagagcaaaacaaaagtaagaccaccgcacagcaagcggccgctgatcttcagacctggaggaggagatatgagggacaattggagaagtgaattatataaatataaagtagtaaaaattgaaccattaggagtagcacccaccaaggcaaagagaagagtggtgcagagagaaaaaagagcagtgggaataggagctttgttccttgggttcttgggagcagcaggaagcactatgggcgcagcgtcaatgacgctgacggtacaggccagacaattattgtctggtatagtgcagcagcagaacaatttgctgagggctattgaggcgcaacagcatctgttgcaactcacagtctggggcatcaagcagctccaggcaagaatcctggctgtggaaagatacctaaaggatcaacagctcctggggatttggggttgctctggaaaactcatttgcaccactgctgtgccttggaatgctagttggagtaataaatctctggaacagatttggaatcacacgacctggatggagtgggacagagaaattaacaattacacaagcttaatacactccttaattgaagaatcgcaaaaccagcaagaaaagaatgaacaagaattattggaattagataaatgggcaagtttgtggaattggtttaacataacaaattggctgtggtatataaaattattcataatgatagtaggaggcttggtaggtttaagaatagtttttgctgtactttctatagtgaatagagttaggcagggatattcaccattatcgtttcagacccacctcccaaccccgaggggacccgacaggcccgaaggaatagaagaagaaggtggagagagagacagagacagatccattcgattagtgaacggatctcgacggtatcggttttaaaagaaaaggggggattggggggtacagtgcaggggaaagaatagtagacataatagcaacagacatacaaactaaagaattacaaaaacaaattacaaaaattcaaaattttatcgattttatttagtctccagaaaaaggggggaatgaaagaccccacctgtaggtttggcaagctagcttaagtaacgccattttgcaaggcatggaaaatacataactgagaatagagaagttcagatcaaggttaggaacagagagacagcagaatatgggccaaacaggatatctgtggtaagcagttcctgccccggctcagggccaagaacagatggtccccagatgcggtcccgccctcagcagtttctagagaaccatcagatgtttccagggtgccccaaggacctgaaatgaccctgtgccttatttgaactaaccaatcagttcgcttctcgcttctgttcgcgcgcttctgctccccgagctcaataaaagagcccacaacccctcactcggcgcgccagtcctccgatagactgcgtcgcccgggtaccgatatcacaagtttgtacaaaaaagctgaacgagaaacgtaaaatgatataaatatcaatatattaaattagattttgcataaaaaacagactacataatactgtaaaacacaacatatccagtcactatggcggccgcattaggcaccccaggctttacactttatgcttccggctcgtataatgtgtggattttgagttaggatccgtcgagattttcaggagctaaggaagctaaaatggagaaaaaaatcactggatataccaccgttgatatatcccaatggcatcgtaaagaacattttgaggcatttcagtcagttgctcaatgtacctataaccagaccgttcagctggatattacggcctttttaaagaccgtaaagaaaaataagcacaagttttatccggcctttattcacattcttgcccgcctgatgaatgctcatccggaattccgtatggcaatgaaagacggtgagctggtgatatgggatagtgttcacccttgttacaccgttttccatgagcaaactgaaacgttttcatcgctctggagtgaataccacgacgatttccggcagtttctacacatatattcgcaagatgtggcgtgttacggtgaaaacctggcctatttccctaaagggtttattgagaatatgtttttcgtctcagccaatccctgggtgagtttcaccagttttgatttaaacgtggccaatatggacaacttcttcgcccccgttttcaccatgggcaaatattatacgcaaggcgacaaggtgctgatgccgctggcgattcaggttcatcatgccgtttgtgatggcttccatgtcggcagaatgcttaatgaattacaacagtactgcgatgagtggcagggcggggcgtaaacgcgtggatccggcttactaaaagccagataacagtatgcgtatttgcgcgctgatttttgcggtataagaatatatactgatatgtatacccgaagtatgtcaaaaagaggtatgctatgaagcagcgtattacagtgacagttgacagcgacagctatcagttgctcaaggcatatatgatgtcaatatctccggtctggtaagcacaaccatgcagaatgaagcccgtcgtctgcgtgccgaacgctggaaagcggaaaatcaggaagggatggctgaggtcgcccggtttattgaaatgaacggctcttttgctgacgagaacaggggctggtgaaatgcagtttaaggtttacacctataaaagagagagccgttatcgtctgtttgtggatgtacagagtgatattattgacacgcccgggcgacggatggtgatccccctggccagtgcacgtctgctgtcagataaagtctcccgtgaactttacccggtggtgcatatcggggatgaaagctggcgcatgatgaccaccgatatggccagtgtgccggtctccgttatcggggaagaagtggctgatctcagccaccgcgaaaatgacatcaaaaacgccattaacctgatgttctggggaatataaatgtcaggctcccttatacacagccagtctgcaggtcgaccatagtgactggatatgttgtgttttacagtattatgtagtctgttttttatgcaaaatctaatttaatatattgatatttatatcattttacgtttctcgttcagctttcttgtacaaagtggtgattcgagttaattaagctagcctagtgccatttgttcagtggttcgtagggctttcccccactgtttggctttcagttatatggatgatgtggtattgggggccaagtctgtacagcatcttgagtccctttttaccgctgttaccaattttcttttgtctttgggtatacatttaaaccctaacaaaacaaagagatggggttactctctaaattttatgggttatgtcattggatgttatgggtccttgccacaagaacacatcatacaaaaaatcaaagaatgttttagaaaacttcctattaacaggcctattgattggaaagtatgtcaacgaattgtgggtcttttgggttttgctgccccttttacacaatgtggttatcctgcgttgatgcctttgtatgcatgtattcaatctaagcaggctttcactttctcgccaacttacaaggcctttctgtgtaaacaatacctgaacctttaccccgttgcccggcaacggccaggtctgtgccaagtgtttgctgacgcaacccccactggctggggcttggtcatgggccatcagcgcatgcgtggaaccttttcggctcctctgccgatccatactgcggaactcctagccgcttgttttgctcgcagcaggtctggagcaaacattatcgggactgataactctgttgtcctatcccgcaaatatacatcgtttccatggctgctaggctgtgctgccaactggatcctgcgcgggacgtcctttgtttacgtcccgtcggcgctgaatcctgcggacgacccttctcggggtcgcttgggactctctcgtccccttctccgtctgccgttccgaccgaccacggggcgcacctctctttacgcggactccccgtctgtgccttctcatctgccggaccgtgtgcacttcgcttcacctctgcacgtcgcatggagaccaccgtgaacgcccaccaaatattgcccaaggtcttacataagaggactcttggactctcagcaatgtcaacgaccgaccttgaggcatacttcaaagactgtttgtttaaagactgggaggagttgggggaggagattaggttaaaggtctttgtactaggaggctgtaggcataaattggtctgcgcaccagcaccatggcgcaatcactagagcggggtacctttaagaccaatgacttacaaggcagctgtagatcttagccactttttaaaagaaaaggggggactggaagggctaattcactcccaacgaagacaagatctgctttttgcttgtactgggtctctctggttagaccagatctgagcctgggagctctctggctaactagggaacccactgcttaagcctcaataaagcttgccttgagtgcttcaagtagtgtgtgcccgtctgttgtgtgactctggtaactagagatccctcagacccttttagtcagtgtggaaaatctctagcagtagtagttcatgtcatcttattattcagtatttataacttgcaaagaaatgaatatcagagagtgagaggaacttgtttattgcagcttataatggttacaaataaagcaatagcatcacaaatttcacaaataaagcatttttttcactgcattctagttgtggtttgtccaaactcatcaatgtatcttatcatgtctggctctagctatcccgcccctaactccgcccatcccgcccctaactccgcccagttccgcccattctccgccccatggctgactaattttttttatttatgcagaggccgaggccggatcccttgagtggctttcatcctggagcagactttgcagtctgtggactgcaacacaacattgcctttatgtgtaactcttggctgaagctcttacaccaatgctgggggacatgtacctcccaggggcccaggaagactacgggaggctacaccaacgtcaatcagaggggcctgtgtagctaccgataagcggaccctcaagagggcattagcaatagtgtttataaggcccccttgttaattcttgaagacgaaagggcctcgtgatacgcctatttttataggttaatgtcatgataataatggtttcttagacgtcaggtggcacttttcggggaaatgtgcgcggaacccctatttgtttatttttctaaatacattcaaatatgtatccgctcatgagacaataaccctgataaatgcttcaataatattgaaaaaggaagagtatgagtattcaacatttccgtgtcgcccttattcccttttttgcggcattttgccttcctgtttttgctcacccagaaacgctggtgaaagtaaaagatgctgaagatcagttgggtgcacgagtgggttacatcgaactggatctcaacagcggtaagatccttgagagttttcgccccgaagaacgttttccaatgatgagcacttttaaagttctgctatgtggcgcggtattatcccgtgttgacgccgggcaagagcaactcggtcgccgcatacactattctcagaatgacttggttgagtactcaccagtcacagaaaagcatcttacggatggcatgacagtaagagaattatgcagtgctgccataaccatgagtgataacactgcggccaacttacttctgacaacgatcggaggaccgaaggagctaaccgcttttttgcacaacatgggggatcatgtaactcgccttgatcgttgggaaccggagctgaatgaagccataccaaacgacgagcgtgacaccacgatgcctgcagcaatggcaacaacgttgcgcaaactattaactggcgaactacttactctagcttcccggcaacaattaatagactggatggaggcggataaagttgcaggaccacttctgcgctcggcccttccggctggctggtttattgctgataaatctggagccggtgagcgtgggtctcgcggtatcattgcagcactggggccagatggtaagccctcccgtatcgtagttatctacacgacggggagtcaggcaactatggatgaacgaaatagacagatcgctgagataggtgcctcactgattaagcattggtaactgtcagaccaagtttactcatatatactttagattgatttaaaacttcatttttaatttaaaaggatctaggtgaagatcctttttgataatctcatgaccaaaatcccttaacgtgagttttcgttccactgagcgtcagaccccgtagaaaagatcaaaggatcttcttgagatcctttttttctgcgcgtaatctgctgcttgcaaacaaaaaaaccaccgctaccagcggtggtttgtttgccggatcaagagctaccaactctttttccgaaggtaactggcttcagcagagcgcagataccaaatactgtccttctagtgtagccgtagttaggccaccacttcaagaactctgtagcaccgcctacatacctcgctctgctaatcctgttaccagtggctgctgccagtggcgataagtcgtgtcttaccgggttggactcaagacgatagttaccggataaggcgcagcggtcgggctgaacggggggttcgtgcacacagcccagcttggagcgaacgacctacaccgaactgagatacctacagcgtgagcattgagaaagcgccacgcttcccgaagggagaaaggcggacaggtatccggtaagcggcagggtcggaacaggagagcgcacgagggagcttccagggggaaacgcctggtatctttatagtcctgtcgggtttcgccacctctgacttgagcgtcgatttttgtgatgctcgtcaggggggcggagcctatggaaaaacgccagcaacgcggcctttttacggttcctggccttttgctggcctttttgaagctgtccctgatggtcgtcatctacctgcctggacagcatggcctgcaacgcgggcatcccgatgccgccggaagcgagaagaatcataatggggaaggccatccagcctcgcgtcg

SEQ ID NO: 36 - DNA, 7298 bp, Artificial Sequence
  pCIGO-VSV.G (VSVG)
gtcgacggatcgggagatcaattccggcacctgtcctacgagttgcatgataaagaagacagtcataagtgcggcgacgatagtcatgccccgcgcccaccggaaggagctgactgggttgaaggctctcaagggcatcggtcgatgcaggaaaaggacaagcagcgaaaattcacgcccccttgggaggtggcggcatatgcaaaggatagcactcccactctactactgggtatcatatgctgactgtatatgcatgaggatagcatatgctacccggatacagattaggatagcatatactacccagatatagattaggatagcatatgctacccagatatagattaggatagcctatgctacccagatataaattaggatagcatatactacccagatatagattaggatagcatatgctacccagatatagattaggatagcctatgctacccagatatagattaggatagcatatgctacccagatatagattaggatagcatatgctatccagatatttgggtagtatatgctacccagatataaattaggatagcatatactaccctaatctctattaggatagcatatgctacccggatacagattaggatagcatatactacccagatatagattaggatagcatatgctacccagatatagattaggatagcctatgctacccagatataaattaggatagcatatactacccagatatagattaggatagcatatgctacccagatatagattaggatagcctatgctacccagatatagattaggatagcatatgctatccagatatttgggtagtatatgctacccatggcaacattagcccaccgtgctctcagcgacctcgtgaatatgaggaccaacaaccctgtgcttggcgctcaggcgcaagtgtgtgtaatttgtcctccagatcgcagcaatcgcgcccctatcttggcccgcccacctacttatgcaggtattccccggggtgccattagtggttttgtgggcaagtggtttgaccgcagtggttagcggggttacaatcagccaagttattacacccttattttacagtccaaaaccgcagggcggcgtgtgggggctgacgcgtgcccccactccacaatttcaaaaaaaagagtggccacttgtctttgtttatgggccccattggcgtggagccccgtttaattttcgggggtgttagagacaaccagtggagtccgctgctgtcggcgtccactctctttccccttgttacaaatagagtgtaacaacatggttcacctgtcttggtccctgcctgggacacatcttaataaccccagtatcatattgcactaggattatgtgttgcccatagccataaattcgtgtgagatggacatccagtctttacggcttgtccccaccccatggatttctattgttaaagatattcagaatgtttcattcctacactagtatttattgcccaaggggtttgtgagggttatattggtgtcatagcacaatgccaccactgaaccccccgtccaaattttattctgggggcgtcacctgaaaccttgttttcgagcacctcacatacaccttactgttcacaactcagcagttattctattagctaaacgaaggagaatgaagaagcaggcgaagattcaggagagttcactgcccgctccttgatcttcagccactgcccttgtgactaaaatggttcactaccctcgtggaatcctgaccccatgtaaataaaaccgtgacagctcatggggtgggagatatcgctgttccttaggacccttttactaaccctaattcgatagcatatgcttcccgttgggtaacatatgctattgaattagggttagtctggatagtatatactactacccgggaagcatatgctacccgtttagggttaacaagggggccttataaacactattgctaatgccctcttgagggtccgcttatcggtagctacacaggcccctctgattgacgttggtgtagcctcccgtagtcttcctgggcccctgggaggtacatgtcccccagcattggtgtaagagcttcagccaagagttacacataaaggcaatgttgtgttgcagtccacagactgcaaagtctgctccaggatgaaagccactcaagggatcttcaatattggccattagccatattattcattggttatatagcataaatcaatattggctattggccattgcatacgttgtatctatatcataatatgtacatttatattggctcatgtccaatatgaccgccatgttggcattgattattgactagttattaatagtaatcaattacggggtcattagttcatagcccatatatggagttccgcgttacataacttacggtaaatggcccgcctggctgaccgcccaacgacccccgcccattgacgtcaataatgacgtatgttcccatagtaacgccaatagggactttccattgacgtcaatgggtggagtatttacggtaaactgcccacttggcagtacatcaagtgtatcatatgccaagtccgccccctattgacgtcaatgacggtaaatggcccgcctggcattatgcccagtacatgaccttacgggactttcctacttggcagtacatctacgtattagtcatcgctattaccatggtgatgcggttttggcagtacaccaatgggcgtggatagcggtttgactcacggggatttccaagtctccaccccattgacgtcaatgggagtttgttttggcaccaaaatcaacgggactttccaaaatgtcgtaataaccccgccccgttgacgcaaatgggcggtaggcgtgtacggtgggaggtctatataagcagagctcgtttagtgaaccgtcagatcactagaagctttattgcggtagtttatcacagttaaattgctaacgcagtcagtgcttctgacacaacagtctcgaacttaagctgcagaagttggtcgtgaggcactgggcaggtaagtatcaaggttacaagacaggtttaaggagaccaatagaaactgggcttgtcgagacagagaagactcttgcgtttctgataggcacctattggtcttactgacatccactttgcctttctctccacaggtgtccactcccagttcaattacagctcttaaggctagagtacttaatacgactcactataggctagcggtaccgagctcggatccactagtaacggccgccagtgtgctggaattcaacagagatcgatctgtttccttgacactatgaagtgccttttgtacttagcctttttattcattggggtgaattgcaagttcaccatagtttttccacacaaccaaaaaggaaactggaaaaatgttccttctaattaccattattgcccgtcaagctcagatttaaattggcataatgacttaataggcacagccatacaagtcaaaatgcccaagagtcacaaggctattcaagcagacggttggatgtgtcatgcttccaaatgggtcactacttgtgatttccgctggtatggaccgaagtatataacacagtccatccgatccttcactccatctgtagaacaatgcaaggaaagcattgaacaaacgaaacaaggaacttggctgaatccaggcttccctcctcaaagttgtggatatgcaactgtgacggatgccgaagcagtgattgtccaggtgactcctcaccatgtgctggttgatgaatacacaggagaatgggttgattcacagttcatcaacggaaaatgcagcaattacatatgccccactgtccataactctacaacctggcattctgactataaggtcaaagggctatgtgattctaacctcatttccatggacatcaccttcttctcagaggacggagagctatcatccctgggaaaggagggcacagggttcagaagtaactactttgcttatgaaactggaggcaaggcctgcaaaatgcaatactgcaagcattggggagtcagactcccatcaggtgtctggttcgagatggctgataaggatctctttgctgcagccagattccctgaatgcccagaagggtcaagtatctctgctccatctcagacctcagtggatgtaagtctaattcaggacgttgagaggatcttggattattccctctgccaagaaacctggagcaaaatcagagcgggtcttccaatctctccagtggatctcagctatcttgctcctaaaaacccaggaaccggtcctgctttcaccataatcaatggtaccctaaaatactttgagaccagatacatcagagtcgatattgctgctccaatcctctcaagaatggtcggaatgatcagtggaactaccacagaaagggaactgtgggatgactgggcaccatatgaagacgtggaaattggacccaatggagttctgaggaccagttcaggatataagtttcctttatacatgattggacatggtatgttggactccgatcttcatcttagctcaaaggctcaggtgttcgaacatcctcacattcaagacgctgcttcgcaacttcctgatgatgagagtttattttttggtgatactgggctatccaaaaatccaatcgagcttgtagaaggttggttcagtagttggaaaagctctattgcctcttttttctttatcatagggttaatcattggactattcttggttctccgagttggtatccatctttgcattaaattaaagcacaccaagaaaagacagatttatacagacatagagatgaaccgacttggaaagtaactcaaatcctgcacaacagattcttcatgtttggaccaaatcaacttgtgataccatgctcaaagaggcctcaattatatttgagtttttaatttttatggaattctgcagatatccatcacactggcggccgctcgagcatgcatctagagggccctattctatagtgtcacctaaatgctagagctcgctgatcagcctcgactgtgccttctagttgccagccatctgttgtttgcccctcccccgtgccttccttgaccctggaaggtgccactcccactgtcctttcctaataaaatgaggaaattgcatcgcattgtctgagtaggtgtcattctattctggggggtggggtggggcaggacagcaagggggaggattgggaagacaatagcaggcatgctggggatgcggtgggctctatggcttctgaggcggaaagaaccagctgcattaatgaatcggccaacgcgcggggagaggcggtttgcgtattgggcgctcttccgcttcctcgctcactgactcgctgcgctcggtcgttcggctgcggcgagcggtatcagctcactcaaaggcggtaatacggttatccacagaatcaggggataacgcaggaaagaacatgtgagcaaaaggccagcaaaaggccaggaaccgtaaaaaggccgcgttgctggcgtttttccataggctccgcccccctgacgagcatcacaaaaatcgacgctcaagtcagaggtggcgaaacccgacaggactataaagataccaggcgtttccccctggaagctccctcgtgcgctctcctgttccgaccctgccgcttaccggatacctgtccgcctttctcccttcgggaagcgtggcgctttctcaatgctcacgctgtaggtatctcagttcggtgtaggtcgttcgctccaagctgggctgtgtgcacgaaccccccgttcagcccgaccgctgcgccttatccggtaactatcgtcttgagtccaacccggtaagacacgacttatcgccactggcagcagccactggtaacaggattagcagagcgaggtatgtaggcggtgctacagagttcttgaagtggtggcctaactacggctacactagaaggacagtatttggtatctgcgctctgctgaagccagttaccttcggaaaaagagttggtagctcttgatccggcaaacaaaccaccgctggtagcggtggtttttttgtttgcaagcagcagattacgcgcagaaaaaaaggatctcaagaagatcctttgatcttttctacggggtctgacgctcagtggaacgaaaactcacgttaagggattttggtcatgagattatcaaaaaggatcttcacctagatccttttaaattaaaaatgaagttttaaatcaatctaaagtatatatgagtaaacttggtctgacagttaccaatgcttaatcagtgaggcacctatctcagcgatctgtctatttcgttcatccatagttgcctgactccccgtcgtgtagataactacgatacgggagggcttaccatctggccccagtgctgcaatgataccgcgagacccacgctcaccggctccagatttatcagcaataaaccagccagccggaagggccgagcgcagaagtggtcctgcaactttatccgcctccatccagtctattaattgttgccgggaagctagagtaagtagttcgccagttaatagtttgcgcaacgttgttgccattgctacaggcatcgtggtgtcacgctcgtcgtttggtatggcttcattcagctccggttcccaacgatcaaggcgagttacatgatcccccatgttgtgcaaaaaagcggttagctccttcggtcctccgatcgttgtcagaagtaagttggccgcagtgttatcactcatggttatggcagcactgcataattctcttactgtcatgccatccgtaagatgcttttctgtgactggtgagtactcaaccaagtcattctgagaatagtgtatgcggcgaccgagttgctcttgcccggcgtcaatacgggataataccgcgccacatagcagaactttaaaagtgctcatcattggaaaacgttcttcggggcgaaaactctcaaggatcttaccgctgttgagatccagttcgatgtaacccactcgtgcacccaactgatcttcagcatcttttactttcaccagcgtttctgggtgagcaaaaacaggaaggcaaaatgccgcaaaaaagggaataagggcgacacggaaatgttgaatactcatactcttcctttttcaatattattgaagcatttatcagggttattgtctcatgagcggatacatatttgaatgtatttagaaaaataaacaaataggggttccgcgcacatttccccgaaaagtgccacctgac

SEQ ID NO: 37 - DNA, 9932 bp, Artificial Sequence
  PLV4301G38A1
cgataaccctaattcgatagcatatgcttcccgttgggtaacatatgctattgaattagggttagtctggatagtatatactactacccgggaagcatatgctacccgtttagggttcaccggtgatgccggccacgatgcgtccggcgtagaggatctaatgtgagttagctcactcattaggcaccccaggctttacactttatgcttccggctcgtatgttgtgtggaattgtgagcggataacaatttcacacaggaaacagctatgaccatgattacgccaagcgcgcaattaaccctcactaaagggaacaaaagctggagctgcaagcttaatgtagtcttatgcaatactcttgtagtcttgcaacatggtaacgatgagttagcaacatgccttacaaggagagaaaaagcaccgtgcatgccgattggtggaagtaaggtggtacgatcgtgccttattaggaaggcaacagacgggtctgacatggattggacgaaccactgaattgccgcattgcagagatattgtatttaagtgcctagctcgatacataaacgggtctctctggttagaccagatctgagcctgggagctctctggctaactagggaacccactgcttaagcctcaataaagcttgccttgagtgcttcaagtagtgtgtgcccgtctgttgtgtgactctggtaactagagatccctcagacccttttagtcagtgtggaaaatctctagcagtggcgcccgaacagggacttgaaagcgaaagggaaaccagaggagctctctcgacgcaggactcggcttgctgaagcgcgcacggcaagaggcgaggggcggcgactggtgagtacgccaaaaattttgactagcggaggctagaaggagagagatgggtgcgagagcgtcagtattaagcgggggagaattagatcgcgatgggaaaaaattcggttaaggccagggggaaagaaaaaatataaattaaaacatatagtatgggcaagcagggagctagaacgattcgcagttaatcctggcctgttagaaacatcagaaggctgtagacaaatactgggacagctacaaccatcccttcagacaggatcagaagaacttagatcattatataatacagtagcaaccctctattgtgtgcatcaaaggatagagataaaagacaccaaggaagctttagacaagatagaggaagagcaaaacaaaagtaagaccaccgcacagcaagcggccgctgatcttcagacctggaggaggagatatgagggacaattggagaagtgaattatataaatataaagtagtaaaaattgaaccattaggagtagcacccaccaaggcaaagagaagagtggtgcagagagaaaaaagagcagtgggaataggagctttgttccttgggttcttgggagcagcaggaagcactatgggcgcagcgtcaatgacgctgacggtacaggccagacaattattgtctggtatagtgcagcagcagaacaatttgctgagggctattgaggcgcaacagcatctgttgcaactcacagtctggggcatcaagcagctccaggcaagaatcctggctgtggaaagatacctaaaggatcaacagctcctggggatttggggttgctctggaaaactcatttgcaccactgctgtgccttggaatgctagttggagtaataaatctctggaacagatttggaatcacacgacctggatggagtgggacagagaaattaacaattacacaagcttaatacactccttaattgaagaatcgcaaaaccagcaagaaaagaatgaacaagaattattggaattagataaatgggcaagtttgtggaattggtttaacataacaaattggctgtggtatataaaattattcataatgatagtaggaggcttggtaggtttaagaatagtttttgctgtactttctatagtgaatagagttaggcagggatattcaccattatcgtttcagacccacctcccaaccccgaggggacccgacaggcccgaaggaatagaagaagaaggtggagagagagacagagacagatccattcgattagtgaacggatctcgacggtatcggttttaaaagaaaaggggggattggggggtacagtgcaggggaaagaatagtagacataatagcaacagacatacaaactaaagaattacaaaaacaaattacaaaaattcaaaattttatcgattttatttagtctccagaaaaaggggggaatgaaagaccccacctgtaggtttggcaagctagcttaagtaacgccattttgcaaggcatggaaaatacataactgagaatagagaagttcagatcaaggttaggaacagagagacagcagaatatgggccaaacaggatatctgtggtaagcagttcctgccccggctcagggccaagaacagatggtccccagatgcggtcccgccctcagcagtttctagagaaccatcagatgtttccagggtgccccaaggacctgaaatgaccctgtgccttatttgaactaaccaatcagttcgcttctcgcttctgttcgcgcgcttctgctccccgagctcaataaaagagcccacaacccctcactcggcgcgccagtcctccgatagactgcgtcgcccgggtaccgatatcaccaactttgtacaaaaaagctgaacgatatcgccaccatgggcagcacagccattctggccctgctgctggcagtgctgcagggcgtgtcagctgaagtgcagctggtggaatctggcggcggactggtgcagcctggcggatctctgagactgagctgtgccgccagcggcttcaccttcagcaactacgccatgagctgggtgcgccaggcccctggaaaaggcctggaatgggtgtccaccatcagcggctctggcggaaccacctactacgccgatagcgtgaagggccggttcaccatctcccgggacaacagcaagaacaccctgtacctgcagatgaacagcctgcgggtggaagataccgccgtgtactactgcgccaaggactggttcagaagcagcagccccgacgccttcgacatctggggccagggaacaaccgtgaccgtgtctgctggcggaggcggatcaggcggcggaggatcagggggaggcggaagcggagcaccttcttacgtgctgacccagccccctagcgtgtcagtggctcctggacagaccgccagaatcacctgtggcggcaacaacatcggccggaagatcgtgcactggtatcagcagaggcccggacaggctcccgtgctcgtgatctactacgacaccgacagacctgccggcatccccgagagattcagcggcagcaacagcggcaacatggccaccctgaccatcagcacagtgggagccggcgacgaggccgactactactgtcaagtgtgggacaccggcagcgatcacgtggtgtttggaggcggcaccaagctgacagtgctgggcccgcgggccaactttgtatacaaaagttgcagcgagagcaagtacggccctccctgccccccttgccctgcccccgagttcctgggcggacccagcgtgttcctgttcccccccaagcccaaggacaccctgatgatcagccggacccccgaggtgacctgtgtggtggtggacgtgtcccaggaggaccccgaggtccagttcaactggtacgtggacggcgtggaggtgcacaacgccaagaccaagccccgggaggagcagttcaatagcacctaccgggtggtgtccgtgctgaccgtgctgcaccaggactggctgaacggcaaggaatacaagtgtaaggtgtccaacaagggcctgcccagcagcatcgagaaaaccatcagcaaggccaagggccagcctcgggagccccaggtgtacaccctgccccctagccaagaggagatgaccaagaatcaggtgtccctgacctgcctggtgaagggcttctaccccagcgacatcgccgtggagtgggagagcaacggccagcccgagaacaactacaagaccaccccccctgtgctggacagcgacggcagcttcttcctgtacagcaggctgaccgtggacaagagccggtggcaggagggcaacgtctttagctgctccgtgatgcacgaggccctgcacaaccactacacccagaagagcctgtccctgagcctgggcaagatgttcagatcttgtgatatttacatctgggcacccttggccggaatctgcgtggcccttctgctgtccttgatcatcactctcatctgctacggctccaccagcggctccggcaagcccggctctggcgagggctccaccagcggcgactacaaggacgacgatgacaagtaataggatatcggttcagctttcttgtacaaagttgggattcgagttaattaagttaacgaattccccccctctccctcccccccccctaacgttactggccgaagccgcttggaataaggccggtgtgcgtttgtctatatgttattttccaccatattgccgtcttttggcaatgtgagggcccggaaacctggccctgtcttcttgacgagcattcctaggggtctttcccctctcgccaaaggaatgcaaggtctgttgaatgtcgtgaaggaagcagttcctctggaagcttcttgaagacaaacaacgtctgtagcgaccctttgcaggcagcggaaccccccacctggcgacaggtgcctctgcggccaaaagccacgtgtataagatacacctgcaaaggcggcacaaccccagtgccacgttgtgagttggatagttgtggaaagagtcaaatggctctcctcaagcgtattcaacaaggggctgaaggatgcccagaaggtaccccattgtatgggatctgatctggggcctcggtgcacatgctttacatgtgtttagtcgaggttaaaaaacgtctaggccccccgaaccacggggacgtggttttcctttgaaaaacacgatgataatatggccacaaccatgggaggcggaagcggcggaggctcccctcgaggcaccatggtgagcaagggcgaggagctgttcaccggggtggtgcccatcctggtcgagctggacggcgacgtaaacggccacaagttcagcgtgtccggcgagggcgagggcgatgccacctacggcaagctgaccctgaagttcatctgcaccaccggcaagctgcccgtgccctggcccaccctcgtgaccaccctgacctacggcgtgcagtgcttcagccgctaccccgaccacatgaagcagcacgacttcttcaagtccgccatgcccgaaggctacgtccaggagcgcaccatcttcttcaaggacgacggcaactacaagacccgcgccgaggtgaagttcgagggcgacaccctggtgaaccgcatcgagctgaagggcatcgacttcaaggaggacggcaacatcctggggcacaagctggagtacaactacaacagccacaacgtctatatcatggccgacaagcagaagaacggcatcaaggtgaacttcaagatccgccacaacatcgaggacggcagcgtgcagctcgccgaccactaccagcagaacacccccatcggcgacggccccgtgctgctgcccgacaaccactacctgagcacccagtccgccctgagcaaagaccccaacgagaagcgcgatcacatggtcctgctggagttcgtgaccgccgccgggatcactctcggcatggacgagctgtacaagtaacgcgtcccgggtctagagctagcggtaccatgcattacgtagtcgacgacttaattaagctagcctagtgccatttgttcagtggttcgtagggctttcccccactgtttggctttcagttatatggatgatgtggtattgggggccaagtctgtacagcatcttgagtccctttttaccgctgttaccaattttcttttgtctttgggtatacatttaaaccctaacaaaacaaagagatggggttactctctaaattttatgggttatgtcattggatgttatgggtccttgccacaagaacacatcatacaaaaaatcaaagaatgttttagaaaacttcctattaacaggcctattgattggaaagtatgtcaacgaattgtgggtcttttgggttttgctgccccttttacacaatgtggttatcctgcgttgatgcctttgtatgcatgtattcaatctaagcaggctttcactttctcgccaacttacaaggcctttctgtgtaaacaatacctgaacctttaccccgttgcccggcaacggccaggtctgtgccaagtgtttgctgacgcaacccccactggctggggcttggtcatgggccatcagcgcatgcgtggaaccttttcggctcctctgccgatccatactgcggaactcctagccgcttgttttgctcgcagcaggtctggagcaaacattatcgggactgataactctgttgtcctatcccgcaaatatacatcgtttccatggctgctaggctgtgctgccaactggatcctgcgcgggacgtcctttgtttacgtcccgtcggcgctgaatcctgcggacgacccttctcggggtcgcttgggactctctcgtccccttctccgtctgccgttccgaccgaccacggggcgcacctctctttacgcggactccccgtctgtgccttctcatctgccggaccgtgtgcacttcgcttcacctctgcacgtcgcatggagaccaccgtgaacgcccaccaaatattgcccaaggtcttacataagaggactcttggactctcagcaatgtcaacgaccgaccttgaggcatacttcaaagactgtttgtttaaagactgggaggagttgggggaggagattaggttaaaggtctttgtactaggaggctgtaggcataaattggtctgcgcaccagcaccatggcgcaatcactagagcggggtacctttaagaccaatgacttacaaggcagctgtagatcttagccactttttaaaagaaaaggggggactggaagggctaattcactcccaacgaagacaagatctgctttttgcttgtactgggtctctctggttagaccagatctgagcctgggagctctctggctaactagggaacccactgcttaagcctcaataaagcttgccttgagtgcttcaagtagtgtgtgcccgtctgttgtgtgactctggtaactagagatccctcagacccttttagtcagtgtggaaaatctctagcagtagtagttcatgtcatcttattattcagtatttataacttgcaaagaaatgaatatcagagagtgagaggaacttgtttattgcagcttataatggttacaaataaagcaatagcatcacaaatttcacaaataaagcatttttttcactgcattctagttgtggtttgtccaaactcatcaatgtatcttatcatgtctggctctagctatcccgcccctaactccgcccatcccgcccctaactccgcccagttccgcccattctccgccccatggctgactaattttttttatttatgcagaggccgaggccggatcccttgagtggctttcatcctggagcagactttgcagtctgtggactgcaacacaacattgcctttatgtgtaactcttggctgaagctcttacaccaatgctgggggacatgtacctcccaggggcccaggaagactacgggaggctacaccaacgtcaatcagaggggcctgtgtagctaccgataagcggaccctcaagagggcattagcaatagtgtttataaggcccccttgttaattcttgaagacgaaagggcctcgtgatacgcctatttttataggttaatgtcatgataataatggtttcttagacgtcaggtggcacttttcggggaaatgtgcgcggaacccctatttgtttatttttctaaatacattcaaatatgtatccgctcatgagacaataaccctgataaatgcttcaataatattgaaaaaggaagagtatgagtattcaacatttccgtgtcgcccttattcccttttttgcggcattttgccttcctgtttttgctcacccagaaacgctggtgaaagtaaaagatgctgaagatcagttgggtgcacgagtgggttacatcgaactggatctcaacagcggtaagatccttgagagttttcgccccgaagaacgttttccaatgatgagcacttttaaagttctgctatgtggcgcggtattatcccgtgttgacgccgggcaagagcaactcggtcgccgcatacactattctcagaatgacttggttgagtactcaccagtcacagaaaagcatcttacggatggcatgacagtaagagaattatgcagtgctgccataaccatgagtgataacactgcggccaacttacttctgacaacgatcggaggaccgaaggagctaaccgcttttttgcacaacatgggggatcatgtaactcgccttgatcgttgggaaccggagctgaatgaagccataccaaacgacgagcgtgacaccacgatgcctgcagcaatggcaacaacgttgcgcaaactattaactggcgaactacttactctagcttcccggcaacaattaatagactggatggaggcggataaagttgcaggaccacttctgcgctcggcccttccggctggctggtttattgctgataaatctggagccggtgagcgtgggtctcgcggtatcattgcagcactggggccagatggtaagccctcccgtatcgtagttatctacacgacggggagtcaggcaactatggatgaacgaaatagacagatcgctgagataggtgcctcactgattaagcattggtaactgtcagaccaagtttactcatatatactttagattgatttaaaacttcatttttaatttaaaaggatctaggtgaagatcctttttgataatctcatgaccaaaatcccttaacgtgagttttcgttccactgagcgtcagaccccgtagaaaagatcaaaggatcttcttgagatcctttttttctgcgcgtaatctgctgcttgcaaacaaaaaaaccaccgctaccagcggtggtttgtttgccggatcaagagctaccaactctttttccgaaggtaactggcttcagcagagcgcagataccaaatactgtccttctagtgtagccgtagttaggccaccacttcaagaactctgtagcaccgcctacatacctcgctctgctaatcctgttaccagtggctgctgccagtggcgataagtcgtgtcttaccgggttggactcaagacgatagttaccggataaggcgcagcggtcgggctgaacggggggttcgtgcacacagcccagcttggagcgaacgacctacaccgaactgagatacctacagcgtgagcattgagaaagcgccacgcttcccgaagggagaaaggcggacaggtatccggtaagcggcagggtcggaacaggagagcgcacgagggagcttccagggggaaacgcctggtatctttatagtcctgtcgggtttcgccacctctgacttgagcgtcgatttttgtgatgctcgtcaggggggcggagcctatggaaaaacgccagcaacgcggcctttttacggttcctggccttttgctggcctttttgaagctgtccctgatggtcgtcatctacctgcctggacagcatggcctgcaacgcgggcatcccgatgccgccggaagcgagaagaatcataatggggaaggccatccagcctcgcgtcg

SEQ ID NO: 38 - DNA, 9932 bp, Artificial Sequence; identical to SEQ ID NO: 37
  PLV4301G19H9

SEQ ID NO: 39 - protein, 330 aa, Artificial Sequence [sequence omitted]

SEQ ID NO: 40 - protein, 326 aa, Artificial Sequence
  IgG2
ASTKGPSVFPLAPCSRSTSESTAALGCLVKDYFPEPVTVSWNSGALTSGVHTFPAVLQSSGLYSLSSVVTVPSSNFGTQTYTCNVDHKPSNTKVDKTVERKCCVECPPCPAPPVAGPSVFLFPPKPKDTLMISRTPEVTCVVVDVSHEDPEVQFNWYVDGVEVHNAKTKPREEQFNSTFRVVSVLTVVHQDWLNGKEYKCKVSNKGLPAPIEKTISKTKGQPREPQVYTLPPSREEMTKNQVSLTCLVKGFYPSDIAVEWESNGQPENNYKTTPPMLDSDGSFFLYSKLTVDKSRWQQGNVFSCSVMHEALHNHYTQKSLSLSPGK

SEQ ID NO: 41 - protein, 377 aa, Artificial Sequence
  IgG3
ASTKGPSVFPLAPCSRSTSGGTAALGCLVKDYFPEPVTVSWNSGALTSGVHTFPAVLQSSGLYSLSSVVTVPSSSLGTQTYTCNVNHKPSNTKVDKRVELKTPLGDTTHTCPRCPEPKSCDTPPPCPRCPEPKSCDTPPPCPRCPEPKSCDTPPPCPRCPAPELLGGPSVFLFPPKPKDTLMISRTPEVTCVVVDVSHEDPEVQFKWYVDGVEVHNAKTKPREEQYNSTFRVVSVLTVLHQDWLNGKEYKCKVSNKALPAPIEKTISKTKGQPREPQVYTLPPSREEMTKNQVSLTCLVKGFYPSDIAVEWESSGQPENNYNTTPPMLDSDGSFFLYSKLTVDKSRWQQGNIFSCSVMHEALHNRFTQKSLSLSPGK

SEQ ID NO: 42 - protein, 327 aa, Artificial Sequence
  IgG4
ASTKGPSVFPLAPCSRSTSESTAALGCLVKDYFPEPVTVSWNSGALTSGVHTFPAVLQSSGLYSLSSVVTVPSSSLGTKTYTCNVDHKPSNTKVDKRVESKYGPPCPSCPAPEFLGGPSVFLFPPKPKDTLMISRTPEVTCVVVDVSQEDPEVQFNWYVDGVEVHNAKTKPREEQFNSTYRVVSVLTVLHQDWLNGKEYKCKVSNKGLPSSIEKTISKAKGQPREPQVYTLPPSQEEMTKNQVSLTCLVKGFYPSDIAVEWESNGQPENNYKTTPPVLDSDGSFFLYSRLTVDKSRWQEGNVFSCSVMHEALHNHYTQKSLSLSLGK